European Patent Application EP 4 227 413 A1, published August 16, 2023. Title: NOVEL ANTI-SUGAR CHAIN ANTIBODIES AND THEIR USES. Applicant: NATIONAL UNIVERSITY CORPORATION CHIBA UNIVERSITY. The sequence listing filed with the application follows.

SEQUENCE LISTING (29 sequences)

SEQ ID NO: 1 - protein, 8 aa, Mus musculus
GFSLTSYA

SEQ ID NO: 2 - protein, 7 aa, Mus musculus
IWGGGST

SEQ ID NO: 3 - protein, 11 aa, Mus musculus
AKHEKLGRFPY

SEQ ID NO: 4 - protein, 5 aa, Mus musculus
SSVSY

SEQ ID NO: 5 - protein, 3 aa, Mus musculus
EIS

SEQ ID NO: 6 - protein, 9 aa, Mus musculus
QQWNYPLAT

SEQ ID NO: 7 - DNA, 24 bp, Mus musculus
gggttttcattaaccagctatgct

SEQ ID NO: 8 - DNA, 21 bp, Mus musculus
atatggggtggtggaagcaca

SEQ ID NO: 9 - DNA, 33 bp, Mus musculus
gccaaacatgaaaaactgggacgttttccttac

SEQ ID NO: 10 - DNA, 15 bp, Mus musculus
tcgagtgtaagttac

SEQ ID NO: 11 - DNA, 9 bp, Mus musculus
gaaatatcc

SEQ ID NO: 12 - DNA, 27 bp, Mus musculus
cagcagtggaattatcctctggccacg

SEQ ID NO: 13 - protein, 117 aa, Mus musculus
QVQLKESGPGLVAPSQSLSITCTVSGFSLTSYAVHWVRQPPGKGLEWLGIIWGGGSTNYNSALMSRLSISKDNSKSQVFLKMNSLQTDDTAMYYCAKHEKLGRFPYWGQGTLVTVSA

SEQ ID NO: 14 - protein, 106 aa, Mus musculus
EIVLTQSPAITAASLGQKVTITCSASSSVSYMHWYQQKSGTSPKPWIYEISKLASGVPARFSGSGSGTSYSLTISSMEAEDAAIYYCQQWNYPLATFGGGTKLEIK

SEQ ID NO: 15 - protein, 117 aa, Artificial Sequence
  Humanized SF1 Heavy Chain Variable Region H1
QVQLQESGPGLVKPSETLSLTCTVSGFSLTSYAVHWVRQPPGKGLEWLGIIWGGGSTNYNSALKSRVTISKDNSKSQVSLKLSSVTAADTAVYYCAKHEKLGRFPYWGQGTLVTVSS

SEQ ID NO: 16 - protein, 117 aa, Artificial Sequence
  Humanized SF1 Heavy Chain Variable Region H2
QVQLQESGPGLVKPSETLSLTCTVSGFSLTSYAVHWIRQPPGKGLEWIGIIWGGGSTNYNSALKSRVTISKDNSKSQVSLKLSSVTAADTAVYYCAKHEKLGRFPYWGQGTLVTVSS

SEQ ID NO: 17 - protein, 117 aa, Artificial Sequence
  Humanized SF1 Heavy Chain Variable Region H3
QVQLVESGGGVVQPGGSLRLSCAVSGFSLTSYAVHWVRQAPGKGLEWLGIIWGGGSTNYNSAVKGRFTISKDNSKSSVYLQMNSLRTEDTALYYCAKHEKLGRFPYWGQGTLVTVSS

SEQ ID NO: 18 - protein, 106 aa, Artificial Sequence
  Humanized SF1 Heavy Chain Variable Region L1
EIQLTQSPSSLSASVGDRVTITCRASSSVSYMHWYQQKPGKAPKPLIYEISKLASGVPSRFSGSGSGTDYTLTISSLQPEDFATYYCQQWNYPLATFGGGTKLEIK

SEQ ID NO: 19 - protein, 106 aa, Artificial Sequence
  Humanized SF1 Heavy Chain Variable Region L2
DIQLTQSPSSLSASVGDRVTITCRASSSVSYMHWYQQKPGKAPKPLIYEISKLASGVPSRFSGSGSGTDYTLTISSLQPEDFATYYCQQWNYPLATFGGGTKLEIK

SEQ ID NO: 20 - protein, 106 aa, Artificial Sequence
  Humanized SF1 Heavy Chain Variable Region L3
EIVLTQSPDFQSVTPKEKVTITCRASSSVSYMHWYQQKPDQSPKPLIYEISKLASGVPSRFSGSGSGTDYTLTINSLEAEDAATYYCQQWNYPLATFGGGTKLEIK

SEQ ID NO: 21 - protein, 251 aa, Artificial Sequence
  Humanized SF1-scFv-H1L1
QVQLQESGPGLVKPSETLSLTCTVSGFSLTSYAVHWVRQPPGKGLEWLGIIWGGGSTNYNSALKSRVTISKDNSKSQVSLKLSSVTAADTAVYYCAKHEKLGRFPYWGQGTLVTVSSGGGGSGGGGSGGGGSEIQLTQSPSSLSASVGDRVTITCRASSSVSYMHWYQQKPGKAPKPLIYEISKLASGVPSRFSGSGSGTDYTLTISSLQPEDFATYYCQQWNYPLATFGGGTKLEIKGLQQGGTHHHHHH

SEQ ID NO: 22 - protein, 251 aa, Artificial Sequence
  Humanized SF1-scFv-H1L2
QVQLQESGPGLVKPSETLSLTCTVSGFSLTSYAVHWVRQPPGKGLEWLGIIWGGGSTNYNSALKSRVTISKDNSKSQVSLKLSSVTAADTAVYYCAKHEKLGRFPYWGQGTLVTVSSGGGGSGGGGSGGGGSDIQLTQSPSSLSASVGDRVTITCRASSSVSYMHWYQQKPGKAPKPLIYEISKLASGVPSRFSGSGSGTDYTLTISSLQPEDFATYYCQQWNYPLATFGGGTKLEIKGLQQGGTHHHHHH

SEQ ID NO: 23 - protein, 251 aa, Artificial Sequence
  Humanized SF1-scFv-H2L1
QVQLQESGPGLVKPSETLSLTCTVSGFSLTSYAVHWIRQPPGKGLEWIGIIWGGGSTNYNSALKSRVTISKDNSKSQVSLKLSSVTAADTAVYYCAKHEKLGRFPYWGQGTLVTVSSGGGGSGGGGSGGGGSEIQLTQSPSSLSASVGDRVTITCRASSSVSYMHWYQQKPGKAPKPLIYEISKLASGVPSRFSGSGSGTDYTLTISSLQPEDFATYYCQQWNYPLATFGGGTKLEIKGLQQGGTHHHHHH

SEQ ID NO: 24 - protein, 251 aa, Artificial Sequence
  Humanized SF1-scFv-H3L3
QVQLVESGGGVVQPGGSLRLSCAVSGFSLTSYAVHWVRQAPGKGLEWLGIIWGGGSTNYNSAVKGRFTISKDNSKSSVYLQMNSLRTEDTALYYCAKHEKLGRFPYWGQGTLVTVSSGGGGSGGGGSGGGGSEIVLTQSPDFQSVTPKEKVTITCRASSSVSYMHWYQQKPDQSPKPLIYEISKLASGVPSRFSGSGSGTDYTLTINSLEAEDAATYYCQQWNYPLATFGGGTKLEIKGLQQGGTHHHHHH

SEQ ID NO: 25 - protein, 447 aa, Artificial Sequence
  Full Length Humanized SF1 Heavy Chain
QVQLQESGPGLVKPSETLSLTCTVSGFSLTSYAVHWVRQPPGKGLEWLGIIWGGGSTNYNSALKSRVTISKDNSKSQVSLKLSSVTAADTAVYYCAKHEKLGRFPYWGQGTLVTVSSASTKGPSVFPLAPSSKSTSGGTAALGCLVKDYFPEPVTVSWNSGALTSGVHTFPAVLQSSGLYSLSSVVTVPSSSLGTQTYICNVNHKPSNTKVDKKVEPKSCDKTHTCPPCPAPELLGGPSVFLFPPKPKDTLMISRTPEVTCVVVDVSHEDPEVKFNWYVDGVEVHNAKTKPREEQYNSTYRVVSVLTVLHQDWLNGKEYKCKVSNKALPAPIEKTISKAKGQPREPQVYTLPPSRDELTKNQVSLTCLVKGFYPSDIAVEWESNGQPENNYKTTPPVLDSDGSFFLYSKLTVDKSRWQQGNVFSCSVMHEALHNHYTQKSLSLSPGK

SEQ ID NO: 26 - protein, 213 aa, Artificial Sequence
  Full Length Humanized SF1 Light Chain
EIQLTQSPSSLSASVGDRVTITCRASSSVSYMHWYQQKPGKAPKPLIYEISKLASGVPSRFSGSGSGTDYTLTISSLQPEDFATYYCQQWNYPLATFGGGTKLEIKRTVAAPSVFIFPPSDEQLKSGTASVVCLLNNFYPREAKVQWKVDNALQSGNSQESVTEQDSKDSTYSLSSTLTLSKADYEKHKVYACEVTHQGLSSPVTKSFNRGEC

SEQ ID NO: 27 - protein, 447 aa, Artificial Sequence
  Full Length Humanized SF1 Heavy Chain IgG1-LALA
QVQLQESGPGLVKPSETLSLTCTVSGFSLTSYAVHWVRQPPGKGLEWLGIIWGGGSTNYNSALKSRVTISKDNSKSQVSLKLSSVTAADTAVYYCAKHEKLGRFPYWGQGTLVTVSSASTKGPSVFPLAPSSKSTSGGTAALGCLVKDYFPEPVTVSWNSGALTSGVHTFPAVLQSSGLYSLSSVVTVPSSSLGTQTYICNVNHKPSNTKVDKKVEPKSCDKTHTCPPCPAPEAAGGPSVFLFPPKPKDTLMISRTPEVTCVVVDVSHEDPEVKFNWYVDGVEVHNAKTKPREEQYNSTYRVVSVLTVLHQDWLNGKEYKCKVSNKALPAPIEKTISKAKGQPREPQVYTLPPSRDELTKNQVSLTCLVKGFYPSDIAVEWESNGQPENNYKTTPPVLDSDGSFFLYSKLTVDKSRWQQGNVFSCSVMHEALHNHYTQKSLSLSPGK

SEQ ID NO: 28 - protein, 444 aa, Artificial Sequence
  Full Length Humanized SF1 Heavy Chain IgG4-SPLE
QVQLQESGPGLVKPSETLSLTCTVSGFSLTSYAVHWVRQPPGKGLEWLGIIWGGGSTNYNSALKSRVTISKDNSKSQVSLKLSSVTAADTAVYYCAKHEKLGRFPYWGQGTLVTVSSASTKGPSVFPLAPCSRSTSESTAALGCLVKDYFPEPVTVSWNSGALTSGVHTFPAVLQSSGLYSLSSVVTVPSSSLGTKTYTCNVDHKPSNTKVDKRVESKYGPPCPPCPAPEFEGGPSVFLFPPKPKDTLMISRTPEVTCVVVDVSQEDPEVQFNWYVDGVEVHNAKTKPREEQFNSTYRVVSVLTVLHQDWLNGKEYKCKVSNKGLPSSIEKTISKAKGQPREPQVYTLPPSQEEMTKNQVSLTCLVKGFYPSDIAVEWESNGQPENNYKTTPPVLDSDGSFFLYSRLTVDKSRWQEGNVFSCSVMHEALHNHYTQKSLSLSLGK

SEQ ID NO: 29 - protein, 15 aa, Artificial Sequence
  G4S Linker
GGGGSGGGGSGGGGS